European Patent Application EP 4 190 808 A1, published June 7, 2023. Title: HUMANIZED ANTIBODY, CHIMERIC ANTIGEN RECEPTOR, NUCLEIC ACID, VECTOR, CELL AND USE. Applicant: SHANGHAI IMMUNOHEAD BIOTECHNOLOGY CO., LTD. The sequence listing filed with the application follows.

SEQUENCE LISTING (30 sequences)

SEQ ID NO: 1 - protein, 5 aa, Artificial
NYWIN

SEQ ID NO: 2 - protein, 17 aa, Artificial
NIYPSYIYTNYNQEFKD

SEQ ID NO: 3 - protein, 12 aa, Artificial
SPYGYDEYGLDY

SEQ ID NO: 4 - protein, 17 aa, Artificial
KSSQSLLNSRNQKNYLT

SEQ ID NO: 5 - protein, 7 aa, Artificial
WASTRES

SEQ ID NO: 6 - protein, 9 aa, Artificial
QNDYVYPLT

SEQ ID NO: 7 - protein, 121 aa, Artificial
QVQLVQSGAEVKKPGASVKLSCKASGYTFTNYWINWVKQAPGQGLEWIGNIYPSYIYTNYNQEFKDKVTLTVDESTSTAYMELSSLRSEDTAVYYCTRSPYGYDEYGLDYWGQGTTVTVSS

SEQ ID NO: 8 - protein, 121 aa, Artificial
QVQLVQSGAEVKKPGASVKVSCKASGYTFTNYWINWVRQAPGQGLEWIGNIYPSYIYTNYNQEFKDKVTLTVDESTSTAYMELSSLRSEDTAVYYCTRSPYGYDEYGLDYWGQGTTVTVSS

SEQ ID NO: 9 - protein, 121 aa, Artificial
QVQLVQSGAEVKKPGASVKVSCKASGYTFTNYWINWVRQAPGQGLEWIGNIYPSYIYTNYNQEFKDRVTLTRDTSISTAYMELSRLRSDDTAVYYCTRSPYGYDEYGLDYWGQGTTVTVSS

SEQ ID NO: 10 - protein, 121 aa, Artificial
QVQLVQSGAEVKKPGASVKVSCKASGYTFTNYWINWVRQAPGQGLEWIGNIYPSYIYTNYAQKFQGRVTLTRDTSTSTVYMELSSLRSEDTAVYYCTRSPYGYDEYGLDYWGQGTTVTVSS

SEQ ID NO: 11 - protein, 121 aa, Artificial
QVQLVQSGAEVKKPGASVKVSCKASGYTFTNYWINWVRQAPGQGLEWIGNIYPSYIYTNYNQEFKDRVTMTRDTSISTAYMELSRLRSDDTAVYYCTRSPYGYDEYGLDYWGQGTTVTVSS

SEQ ID NO: 12 - protein, 113 aa, Artificial
DIQLTQSPSSLSASVGDRVTMTCKSSQSLLNSRNQKNYLTWYQQKPGKAPKLLIYWASTRESGVPSRFSGSGSGTDFTLTISSVQPEDFATYYCQNDYVYPLTFGQGTKLEIK

SEQ ID NO: 13 - protein, 113 aa, Artificial
DIQLTQSPSSLSASVGDRVTMTCKSSQSLLNTRNQKNYLTWYQQKPGKAPKLLIYWASTRESGVPSRFSGSGSGTDFTLTISSLQPEDFATYYCQNDYVYPLTFGQGTKLEIK

SEQ ID NO: 14 - protein, 113 aa, Artificial
DIVLTQSPDSLAVSLGERATMNCKSSQSLLNSRNQKNYLTWYQQKPGQPPKLLIYWASTRESGVPDRFSGSGSGTDFTLTISSLQAEDVAVYYCQNDYVYPLTFGQGTKLEIK

SEQ ID NO: 15 - protein, 113 aa, Artificial
EIVLTQSPATLSLSPGERATMSCKSSQSLLNSRNQKNYLTWYQQKPGQAPRLLIYWASTRESGIPARFSGSGSGTDFTLTISSLEPEDFAVYYCQNDYVYPLTFGQGTKLEIK

SEQ ID NO: 16 - protein, 121 aa, Artificial
QVKLQQSGAELVRPGASVKLSCKASGYTFTNYWINWVKQRPGQGLEWIGNIYPSYIYTNYNQEFKDKVTLTVDESSSTAYMQLSSPTSEDSAVYYCTRSPYGYDEYGLDYWGQGTTVTVSS

SEQ ID NO: 17 - protein, 113 aa, Artificial
DIELTQSPSSLTVTAGEKVTMNCKSSQSLLNSRNQKNYLTWYQQKPGQPPKLLIYWASTRESGVPDRFTGSGSGTDFTLTISSVQAEDLAVYYCQNDYVYPLTFGAGTKLEIK

SEQ ID NO: 18 - protein, 490 aa, Artificial
MLLLVTSLLLCELPHPAFLLIPQVQLVQSGAEVKKPGASVKLSCKASGYTFTNYWINWVKQAPGQGLEWIGNIYPSYIYTNYNQEFKDKVTLTVDESTSTAYMELSSLRSEDTAVYYCTRSPYGYDEYGLDYWGQGTTVTVSSGGGGSGGGGSGGGGSDIQLTQSPSSLSASVGDRVTMTCKSSQSLLNSRNQKNYLTWYQQKPGKAPKLLIYWASTRESGVPSRFSGSGSGTDFTLTISSVQPEDFATYYCQNDYVYPLTFGQGTKLEIKIEVMYPPPYLDNEKSNGTIIHVKGKHLCPSPLFPGPSKPFWVLVVVGGVLACYSLLVTVAFIIFWVRSKRSRLLHSDYMNMTPRRPGPTRKHYQPYAPPRDFAAYRSRVKFSRSADAPAYQQGQNQLYNELNLGRREEYDVLDKRRGRDPEMGGKPRRKNPQEGLYNELQKDKMAEAYSEIGMKGERRRGKGHDGLYQGLSTATKDTYDALHMQALPPR

SEQ ID NO: 19 - protein, 490 aa, Artificial
MLLLVTSLLLCELPHPAFLLIPQVQLVQSGAEVKKPGASVKVSCKASGYTFTNYWINWVRQAPGQGLEWIGNIYPSYIYTNYNQEFKDKVTLTVDESTSTAYMELSSLRSEDTAVYYCTRSPYGYDEYGLDYWGQGTTVTVSSGGGGSGGGGSGGGGSDIQLTQSPSSLSASVGDRVTMTCKSSQSLLNSRNQKNYLTWYQQKPGKAPKLLIYWASTRESGVPSRFSGSGSGTDFTLTISSVQPEDFATYYCQNDYVYPLTFGQGTKLEIKIEVMYPPPYLDNEKSNGTIIHVKGKHLCPSPLFPGPSKPFWVLVVVGGVLACYSLLVTVAFIIFWVRSKRSRLLHSDYMNMTPRRPGPTRKHYQPYAPPRDFAAYRSRVKFSRSADAPAYQQGQNQLYNELNLGRREEYDVLDKRRGRDPEMGGKPRRKNPQEGLYNELQKDKMAEAYSEIGMKGERRRGKGHDGLYQGLSTATKDTYDALHMQALPPR

SEQ ID NO: 20 - protein, 490 aa, Artificial
MLLLVTSLLLCELPHPAFLLIPQVQLVQSGAEVKKPGASVKVSCKASGYTFTNYWINWVRQAPGQGLEWIGNIYPSYIYTNYNQEFKDRVTLTRDTSISTAYMELSRLRSDDTAVYYCTRSPYGYDEYGLDYWGQGTTVTVSSGGGGSGGGGSGGGGSDIQLTQSPSSLSASVGDRVTMTCKSSQSLLNSRNQKNYLTWYQQKPGKAPKLLIYWASTRESGVPSRFSGSGSGTDFTLTISSVQPEDFATYYCQNDYVYPLTFGQGTKLEIKIEVMYPPPYLDNEKSNGTIIHVKGKHLCPSPLFPGPSKPFWVLVVVGGVLACYSLLVTVAFIIFWVRSKRSRLLHSDYMNMTPRRPGPTRKHYQPYAPPRDFAAYRSRVKFSRSADAPAYQQGQNQLYNELNLGRREEYDVLDKRRGRDPEMGGKPRRKNPQEGLYNELQKDKMAEAYSEIGMKGERRRGKGHDGLYQGLSTATKDTYDALHMQALPPR

SEQ ID NO: 21 - protein, 490 aa, Artificial
MLLLVTSLLLCELPHPAFLLIPQVQLVQSGAEVKKPGASVKVSCKASGYTFTNYWINWVRQAPGQGLEWIGNIYPSYIYTNYNQEFKDRVTLTRDTSISTAYMELSRLRSDDTAVYYCTRSPYGYDEYGLDYWGQGTTVTVSSGGGGSGGGGSGGGGSDIQLTQSPSSLSASVGDRVTMTCKSSQSLLNTRNQKNYLTWYQQKPGKAPKLLIYWASTRESGVPSRFSGSGSGTDFTLTISSLQPEDFATYYCQNDYVYPLTFGQGTKLEIKIEVMYPPPYLDNEKSNGTIIHVKGKHLCPSPLFPGPSKPFWVLVVVGGVLACYSLLVTVAFIIFWVRSKRSRLLHSDYMNMTPRRPGPTRKHYQPYAPPRDFAAYRSRVKFSRSADAPAYQQGQNQLYNELNLGRREEYDVLDKRRGRDPEMGGKPRRKNPQEGLYNELQKDKMAEAYSEIGMKGERRRGKGHDGLYQGLSTATKDTYDALHMQALPPR

SEQ ID NO: 22 - protein, 490 aa, Artificial
MLLLVTSLLLCELPHPAFLLIPQVQLVQSGAEVKKPGASVKVSCKASGYTFTNYWINWVRQAPGQGLEWIGNIYPSYIYTNYAQKFQGRVTLTRDTSTSTVYMELSSLRSEDTAVYYCTRSPYGYDEYGLDYWGQGTTVTVSSGGGGSGGGGSGGGGSDIQLTQSPSSLSASVGDRVTMTCKSSQSLLNSRNQKNYLTWYQQKPGKAPKLLIYWASTRESGVPSRFSGSGSGTDFTLTISSVQPEDFATYYCQNDYVYPLTFGQGTKLEIKIEVMYPPPYLDNEKSNGTIIHVKGKHLCPSPLFPGPSKPFWVLVVVGGVLACYSLLVTVAFIIFWVRSKRSRLLHSDYMNMTPRRPGPTRKHYQPYAPPRDFAAYRSRVKFSRSADAPAYQQGQNQLYNELNLGRREEYDVLDKRRGRDPEMGGKPRRKNPQEGLYNELQKDKMAEAYSEIGMKGERRRGKGHDGLYQGLSTATKDTYDALHMQALPPR

SEQ ID NO: 23 - protein, 490 aa, Artificial
MLLLVTSLLLCELPHPAFLLIPQVQLVQSGAEVKKPGASVKVSCKASGYTFTNYWINWVRQAPGQGLEWIGNIYPSYIYTNYNQEFKDRVTMTRDTSISTAYMELSRLRSDDTAVYYCTRSPYGYDEYGLDYWGQGTTVTVSSGGGGSGGGGSGGGGSDIQLTQSPSSLSASVGDRVTMTCKSSQSLLNSRNQKNYLTWYQQKPGKAPKLLIYWASTRESGVPSRFSGSGSGTDFTLTISSVQPEDFATYYCQNDYVYPLTFGQGTKLEIKIEVMYPPPYLDNEKSNGTIIHVKGKHLCPSPLFPGPSKPFWVLVVVGGVLACYSLLVTVAFIIFWVRSKRSRLLHSDYMNMTPRRPGPTRKHYQPYAPPRDFAAYRSRVKFSRSADAPAYQQGQNQLYNELNLGRREEYDVLDKRRGRDPEMGGKPRRKNPQEGLYNELQKDKMAEAYSEIGMKGERRRGKGHDGLYQGLSTATKDTYDALHMQALPPR

SEQ ID NO: 24 - protein, 490 aa, Artificial
MLLLVTSLLLCELPHPAFLLIPQVQLVQSGAEVKKPGASVKVSCKASGYTFTNYWINWVRQAPGQGLEWIGNIYPSYIYTNYNQEFKDKVTLTVDESTSTAYMELSSLRSEDTAVYYCTRSPYGYDEYGLDYWGQGTTVTVSSGGGGSGGGGSGGGGSDIQLTQSPSSLSASVGDRVTMTCKSSQSLLNTRNQKNYLTWYQQKPGKAPKLLIYWASTRESGVPSRFSGSGSGTDFTLTISSLQPEDFATYYCQNDYVYPLTFGQGTKLEIKIEVMYPPPYLDNEKSNGTIIHVKGKHLCPSPLFPGPSKPFWVLVVVGGVLACYSLLVTVAFIIFWVRSKRSRLLHSDYMNMTPRRPGPTRKHYQPYAPPRDFAAYRSRVKFSRSADAPAYQQGQNQLYNELNLGRREEYDVLDKRRGRDPEMGGKPRRKNPQEGLYNELQKDKMAEAYSEIGMKGERRRGKGHDGLYQGLSTATKDTYDALHMQALPPR

SEQ ID NO: 25 - protein, 490 aa, Artificial
MLLLVTSLLLCELPHPAFLLIPQVQLVQSGAEVKKPGASVKVSCKASGYTFTNYWINWVRQAPGQGLEWIGNIYPSYIYTNYNQEFKDKVTLTVDESTSTAYMELSSLRSEDTAVYYCTRSPYGYDEYGLDYWGQGTTVTVSSGGGGSGGGGSGGGGSDIVLTQSPDSLAVSLGERATMNCKSSQSLLNSRNQKNYLTWYQQKPGQPPKLLIYWASTRESGVPDRFSGSGSGTDFTLTISSLQAEDVAVYYCQNDYVYPLTFGQGTKLEIKIEVMYPPPYLDNEKSNGTIIHVKGKHLCPSPLFPGPSKPFWVLVVVGGVLACYSLLVTVAFIIFWVRSKRSRLLHSDYMNMTPRRPGPTRKHYQPYAPPRDFAAYRSRVKFSRSADAPAYQQGQNQLYNELNLGRREEYDVLDKRRGRDPEMGGKPRRKNPQEGLYNELQKDKMAEAYSEIGMKGERRRGKGHDGLYQGLSTATKDTYDALHMQALPPR

SEQ ID NO: 26 - protein, 490 aa, Artificial
MLLLVTSLLLCELPHPAFLLIPQVQLVQSGAEVKKPGASVKVSCKASGYTFTNYWINWVRQAPGQGLEWIGNIYPSYIYTNYNQEFKDKVTLTVDESTSTAYMELSSLRSEDTAVYYCTRSPYGYDEYGLDYWGQGTTVTVSSGGGGSGGGGSGGGGSEIVLTQSPATLSLSPGERATMSCKSSQSLLNSRNQKNYLTWYQQKPGQAPRLLIYWASTRESGIPARFSGSGSGTDFTLTISSLEPEDFAVYYCQNDYVYPLTFGQGTKLEIKIEVMYPPPYLDNEKSNGTIIHVKGKHLCPSPLFPGPSKPFWVLVVVGGVLACYSLLVTVAFIIFWVRSKRSRLLHSDYMNMTPRRPGPTRKHYQPYAPPRDFAAYRSRVKFSRSADAPAYQQGQNQLYNELNLGRREEYDVLDKRRGRDPEMGGKPRRKNPQEGLYNELQKDKMAEAYSEIGMKGERRRGKGHDGLYQGLSTATKDTYDALHMQALPPR

SEQ ID NO: 27 - protein, 490 aa, Artificial
MLLLVTSLLLCELPHPAFLLIPQVQLVQSGAEVKKPGASVKVSCKASGYTFTNYWINWVRQAPGQGLEWIGNIYPSYIYTNYNQEFKDRVTLTRDTSISTAYMELSRLRSDDTAVYYCTRSPYGYDEYGLDYWGQGTTVTVSSGGGGSGGGGSGGGGSDIVLTQSPDSLAVSLGERATMNCKSSQSLLNSRNQKNYLTWYQQKPGQPPKLLIYWASTRESGVPDRFSGSGSGTDFTLTISSLQAEDVAVYYCQNDYVYPLTFGQGTKLEIKIEVMYPPPYLDNEKSNGTIIHVKGKHLCPSPLFPGPSKPFWVLVVVGGVLACYSLLVTVAFIIFWVRSKRSRLLHSDYMNMTPRRPGPTRKHYQPYAPPRDFAAYRSRVKFSRSADAPAYQQGQNQLYNELNLGRREEYDVLDKRRGRDPEMGGKPRRKNPQEGLYNELQKDKMAEAYSEIGMKGERRRGKGHDGLYQGLSTATKDTYDALHMQALPPR

SEQ ID NO: 28 - protein, 490 aa, Artificial
MLLLVTSLLLCELPHPAFLLIPQVQLVQSGAEVKKPGASVKLSCKASGYTFTNYWINWVKQAPGQGLEWIGNIYPSYIYTNYNQEFKDKVTLTVDESTSTAYMELSSLRSEDTAVYYCTRSPYGYDEYGLDYWGQGTTVTVSSGGGGSGGGGSGGGGSEIVLTQSPATLSLSPGERATMSCKSSQSLLNSRNQKNYLTWYQQKPGQAPRLLIYWASTRESGIPARFSGSGSGTDFTLTISSLEPEDFAVYYCQNDYVYPLTFGQGTKLEIKIEVMYPPPYLDNEKSNGTIIHVKGKHLCPSPLFPGPSKPFWVLVVVGGVLACYSLLVTVAFIIFWVRSKRSRLLHSDYMNMTPRRPGPTRKHYQPYAPPRDFAAYRSRVKFSRSADAPAYQQGQNQLYNELNLGRREEYDVLDKRRGRDPEMGGKPRRKNPQEGLYNELQKDKMAEAYSEIGMKGERRRGKGHDGLYQGLSTATKDTYDALHMQALPPR

SEQ ID NO: 29 - protein, 490 aa, Artificial
MLLLVTSLLLCELPHPAFLLIPQVQLVQSGAEVKKPGASVKLSCKASGYTFTNYWINWVKQAPGQGLEWIGNIYPSYIYTNYNQEFKDKVTLTVDESTSTAYMELSSLRSEDTAVYYCTRSPYGYDEYGLDYWGQGTTVTVSSGGGGSGGGGSGGGGSDIVLTQSPDSLAVSLGERATMNCKSSQSLLNSRNQKNYLTWYQQKPGQPPKLLIYWASTRESGVPDRFSGSGSGTDFTLTISSLQAEDVAVYYCQNDYVYPLTFGQGTKLEIKIEVMYPPPYLDNEKSNGTIIHVKGKHLCPSPLFPGPSKPFWVLVVVGGVLACYSLLVTVAFIIFWVRSKRSRLLHSDYMNMTPRRPGPTRKHYQPYAPPRDFAAYRSRVKFSRSADAPAYQQGQNQLYNELNLGRREEYDVLDKRRGRDPEMGGKPRRKNPQEGLYNELQKDKMAEAYSEIGMKGERRRGKGHDGLYQGLSTATKDTYDALHMQALPPR

SEQ ID NO: 30 - protein, 15 aa, Artificial
GGGGSGGGGSGGGGS